European Patent Application EP 4 170 021 A1, published April 26, 2023. Title: MOUSE MCR-1 PROTEIN-RESISTANT HYBRIDOMA CELL LINE, AND MONOCLONAL ANTIBODY (mAb) AND USE THEREOF. Applicant: Tianjin Era Biology Technology Co., Ltd. The sequence listing filed with the application follows.

SEQUENCE LISTING (20 sequences)

SEQ ID NO: 1 - protein, 16 aa, Artificial sequence
RSSQNIVCSYGNPCLE

SEQ ID NO: 2 - protein, 7 aa, Artificial sequence
KVSNRFS

SEQ ID NO: 3 - protein, 9 aa, Artificial sequence
FQGSHVPWT

SEQ ID NO: 4 - protein, 10 aa, Artificial sequence
GYTFTNYIMH

SEQ ID NO: 5 - protein, 17 aa, Artificial sequence
YINPYNDGTKYNEKFKG

SEQ ID NO: 6 - protein, 10 aa, Artificial sequence
GPYGNYAMDY

SEQ ID NO: 7 - protein, 113 aa, Artificial sequence
DVLMTQTPLSLPVSLGDQASISCRSSQNIVCSYGNPCLEWYLQKPGQSPKLLIYKVSNRFSGVPDRFSGSGSGTDFTLKISRVEAEDLGVYYCFQGSHVPWTFGGGTELEIKR

SEQ ID NO: 8 - DNA, 339 bp, Artificial sequence
gatgttttgatgacccagacgccactctccctgcctgtcagtcttggagatcaagcctccatctcttgcagatctagtcagaacattgtatgtagttatggaaacccctgtttagaatggtacctgcagaaaccaggccagtctccaaagctcctgatctacaaagtttccaaccgattttctggggtcccagacaggttcagtggcagtggatcagggacagatttcacactcaagatcagcagagtggaggctgaggatctgggagtttattactgctttcaaggttcacatgttccgtggacgttcggtggaggcaccgagctggaaatcaaacgg

SEQ ID NO: 9 - protein, 118 aa, Artificial sequence
VQLQQSGPELVKPGASVKMSCRASGYTFTNYIMHWVKQKPGQGLDWIGYINPYNDGTKYNEKFKGKATLSSDKSSGTAYMDLSSLTSEDSAVYYCARGPYGNYAMDYWGQGTSVTVSS

SEQ ID NO: 10 - DNA, 354 bp, Artificial sequence
gtgcagcttcagcaatcaggacctgagctggtaaagcctggggcttcagtgaagatgtcctgcagggcttctggatacacattcactaactatattatgcactgggtgaagcagaagcctgggcagggccttgattggattggatatattaatccttacaatgatggtactaagtacaatgagaagttcaaaggcaaggccacactgtcttcagacaaatcctccggcacagcctatatggacctcagcagcctgacctctgaggactctgcggtctattactgtgcgagaggcccctatggtaactatgctatggactactggggtcaaggaacctcagtcaccgtctcttca

SEQ ID NO: 11 - protein, 11 aa, Artificial sequence
RASQDISNYLN

SEQ ID NO: 12 - protein, 7 aa, Artificial sequence
YTSRLHS

SEQ ID NO: 13 - protein, 9 aa, Artificial sequence
QQGDMIPDT

SEQ ID NO: 14 - protein, 10 aa, Artificial sequence
GYAFTSCNMY

SEQ ID NO: 15 - protein, 17 aa, Artificial sequence
YFDPYSGDAYYNQKFKD

SEQ ID NO: 16 - protein, 10 aa, Artificial sequence
WLQLYYALDY

SEQ ID NO: 17 - protein, 114 aa, Artificial sequence
AIQMTQTPSSLSASLGDRVTISCRASQDISNYLNWYQQKPDGTVKLLIYYTSRLHSGVPSRFSGSGSGTDYSLNISNLEQEDFATYFCQQGDMIPDTFGGGTKLEIKRADAAPT

SEQ ID NO: 18 - DNA, 342 bp, Artificial sequence
gctatccagatgacacagactccatcctccctgtctgcctctctgggagacagagtcaccatcagttgcagggcaagtcaggacattagcaattatttaaactggtatcagcagaaaccagatggaactgttaaactcctgatctactacacatcaagattacactcaggagtcccatcaaggttcagtggcagtgggtctggaacagattattctctcaacattagcaacctggagcaggaagattttgccacttacttttgccaacagggtgatatgattccggacacgttcggaggggggaccaaactggaaataaaacgggctgatgctgcaccaact

SEQ ID NO: 19 - protein, 122 aa, Artificial sequence
VKLQQSGPELVKPGASVKVSCKASGYAFTSCNMYWVKQSHGKSLEWIGYFDPYSGDAYYNQKFKDKATLTVDKSSSTAYMHLNSLTSEDSAVYYCASWLQLYYALDYWGQGTSVTVSAAKTT

SEQ ID NO: 20 - DNA, 366 bp, Artificial sequence
gtgaagctgcagcaatctggacctgagctggtgaagcctggggcctcagtgaaggtctcctgcaaggcttctggttatgcattcactagctgcaacatgtactgggtgaaacagagccatggaaagagccttgagtggattggatattttgatccttacagtggtgatgcttactacaaccagaagttcaaggacaaggccacattgactgttgacaagtcctccagcacagcctacatgcatctcaacagcctgacatctgaggactctgcagtctattactgtgcaagttggttacaactttactatgctctagactactggggtcaaggaacctcagtcaccgtctccgcagccaaaacgaca